European Patent Specification EP 4 052 762 B1, published August 27, 2025. Title: Method for Screening malodor masking agents. Applicant: Takasago International Corporation. The sequence listing filed with the application follows.

SEQUENCE LISTING (6 sequences)

SEQ ID NO: 1 - DNA, 1418 bp, Homo sapiens
  CDS (53)..(991)
ttccagcagcttgcgctaaatgaattcatcaagtgactgaagacaaccagtgatggacggggtgaatgatagctccttgcagggctttgttctgatgggcatatcagaccatccccagctggagatgatcttttttatagccatcctcttctcctatttgctgaccctacttgggaactcaaccatcatcttgctttcccgcctggaggcccggctccatacacccatgtacttcttcctcagcaacctctcctccttggaccttgctttcgctactagttcagtcccccaaatgctgatcaatttatggggaccaggcaagaccatcagctatggtggctgcataacccagctctatgtcttcctttggctgggggccaccgagtgcatcctgctggtggtgatggcatttgaccgctacgtggcagtgtgccggcccctccgctacaccgccatcatgaacccccagctctgctggctgctggctgtgattgcctgcctgggtggcttgggcaactctgtgatccagtcaacattcactctgcagctcccattgtgtgggcaccggagggtggagggattcctctgcgaggtgcctgccatgatcaaactggcctgtggcgacacaagtctcaaccaggctgtgctcaatggtgtctgcaccttcttcactgcagtcccactaagcatcatcgtgatctcctactgcctcattgctcaggcagtgctgaaaatccgctctgcagaggggaggcgaaaggcgttcaatacgtgcctctcccatctgctggtggtgttcctcttctatggctcagccagctatgggtatctgcttccggccaagaacagcaaacaggaccagggcaagttcatttccctgttctactcgttggtcacacccatggtgaatcccctcatctacacgctgcggaacatggaagtgaagggcgcactgaggaggttgctggggaaaggaagagaagttggctgagagaacactccttcgttatttattgcgtcttcatctctacatgcgtttctcattaactctctctggccaggtgaacatgaggaatactaattccggtaaaaccaaggcatgttcctgacagccctaagctgacagccctaagctgttgggaacatggttagtgttattcgtaatgttctacacttatttaccaaaaatcctactgtggactaccgatagcaggggagacatgttgttgagggctcagaggttattgacctgtgacagacctgtctcactgtctctgtctctgttgcccacatgttatttaatatgccttatatttctgcagaattctgtacttttctaagcaaagcacctccacttgcagtatcttacataatgttactataattccataaaatcaagccatgtattattaacttca

SEQ ID NO: 2 - protein, 312 aa, Homo sapiens
MDGVNDSSLQGFVLMGISDHPQLEMIFFIAILFSYLLTLLGNSTIILLSRLEARLHTPMYFFLSNLSSLDLAFATSSVPQMLINLWGPGKTISYGGCITQLYVFLWLGATECILLVVMAFDRYVAVCRPLRYTAIMNPQLCWLLAVIACLGGLGNSVIQSTFTLQLPLCGHRRVEGFLCEVPAMIKLACGDTSLNQAVLNGVCTFFTAVPLSIIVISYCLIAQAVLKIRSAEGRRKAFNTCLSHLLVVFLFYGSASYGYLLPAKNSKQDQGKFISLFYSLVTPMVNPLIYTLRNMEVKGALRRLLGKGREVG

SEQ ID NO: 3 - DNA, 942 bp, Homo sapiens
  CDS (1)..(942)
atgaaaaaagaacaagattctaatgtgacagaatttgttcttctgggcctatcatcttcttgggagctgcagctatttctcttcttactatttttgtttttttacattgctattgtcctgggaaacctcttgatagtggtaacagtgcaagcccatgctcacctgctccaatctcctatgtattattttttaggtcatctctctttcattgacctatgcctgagctgtgttactgtgccaaagatgttaggggatttcctacagcagggcaagagcatctctttttcaggatgcctggcccagatctacttcctccactttctaggagccagtgagatgtttttgctgacagtcatggcctatgacaggtatgttgccatctgtaaccctttgcgctaccttacagtcatgaacccccagctatgcctttggttggttcttgcctgctggtgtgggggttttatccactctatcatgcaggtcatactagtcatccagctgcctttctgtgggcccaatgaactggacaacttctactgtgatgtcccacaagtcatcaagctggcctgcatggacacctatgtggtagaggtgctggtgatagccaacagtggtctgctgtctcttgtctgcttcttggtcttactattctcttatgctatcatcctgatcaccctgagaacacacttctgccagggccagaacaaggtcttctctacctgtgcttctcacctgacagtggtcagcctgatcttcgtgccatgcgtattcatctatttgaggcctttctgcagcttctctgtggataagatattctccttgttttacacagtgattacacctatgttgaaccccctcatctacacactcagaaatactgatatgaagacagctatgaagaagctgaggataaaaccatgtggcattccattgccttgttaa

SEQ ID NO: 4 - protein, 313 aa, Homo sapiens
MKKEQDSNVTEFVLLGLSSSWELQLFLFLLFLFFYIAIVLGNLLIVVTVQAHAHLLQSPMYYFLGHLSFIDLCLSCVTVPKMLGDFLQQGKSISFSGCLAQIYFLHFLGASEMFLLTVMAYDRYVAICNPLRYLTVMNPQLCLWLVLACWCGGFIHSIMQVILVIQLPFCGPNELDNFYCDVPQVIKLACMDTYVVEVLVIANSGLLSLVCFLVLLFSYAIILITLRTHFCQGQNKVFSTCASHLTVVSLIFVPCVFIYLRPFCSFSVDKIFSLFYTVITPMLNPLIYTLRNTDMKTAMKKLRIKPCGIPLPC

SEQ ID NO: 5 - DNA, 2445 bp, Bos taurus
  CDS (1)..(1047)
atgaacgggaccgagggcccaaacttctacgtgcctttctccaacaagacgggcgtggtgcgcagccccttcgaggccccgcagtactacctggcggagccatggcagttctccatgctggccgcctacatgttcctgctgatcatgcttggcttccccatcaacttcctcacgctgtacgtcacagtccagcacaagaagctgcgcacacccctcaactacatcctgctcaacctggccgtggccgacctcttcatggtcttcgggggcttcaccaccaccctctacacctctctgcacggatacttcgtctttgggcccacgggctgcaacctggagggcttctttgccaccctgggcggtgaaattgcactgtggtccttggtggtcctggccatcgagcggtacgtggtggtgtgcaagcccatgagcaacttccgcttcggggagaaccacgccatcatgggcgtcgccttcacctgggtcatggctctggcctgtgccgcgccccccctcgtcggctggtccaggtacatcccggagggcatgcagtgctcgtgcgggattgactactacacgccccacgaggagaccaacaatgagtcgttcgtcatctacatgttcgtggtccacttcatcatccccctgattgtcatattcttctgctacgggcagctggtgttcaccgtcaaggaggcggctgcccagcagcaggagtcggccaccactcagaaggccgagaaggaggtcacccgcatggtgatcatcatggtcatcgctttcctaatctgctggctgccctacgctggggtggcgttctacatcttcacccatcagggctctgactttggccccatcttcatgaccatcccggctttctttgccaagacttctgccgtctacaaccccgtcatctacatcatgatgaacaagcagttccggaactgcatggtcaccactctctgctgtggcaagaacccgctgggtgacgacgaggcctccaccaccgtctccaagacagagaccagccaggtggcgcctgcctaagcccctccagggactccgtggccagctgcaggagtccctcagcccccaccccaccccagcctcagcagctccatcaggagccgcgcctgtcggaaccagctctcacaggctccctgagtgtaaacacaaagaccaaccaaccaaatgcaaaagaatcaacgagagaaacaggaggcgcctcacgtggcaggggcggcccgatctggagtcctgatttcccgggggcccgctgtagatccactccccccagctcatctctcagctacacaagagctcttgctctggaaaagtgtcccagcttagggataagtgagtagcacatgacggggcatgccgtaggtgcttattaataaatgctaggtggaggaaagaaggaatgaatggagagatgaacgggtcgggagggcataggcatcctcttacaacatgttagcagcagcagcagcagctcgcccttggctcatgaccttgagcagctgttttgtccttgggcctcactttcttcccccatacaatgggaattccaaatctctcctcacacgggctgctgggaagatcaaatgagattgtgtgtgtgtgcgtgcgtgcgtgctcgcttgtgtgagctctttgtaaatagtaaggagctggacagactgtagttaacattatgaataatatcaagtaatataagtaattcatctcctatgatcatctcctcttgatagcgaccactttgagactgggcaaggctctaagcatccagcctcgtcaggcttataaacattagacagatggcaaggtcagaccagcgccgggtggtgggccacagggaaggacggtcaaggaaatgcagagtgcaggcatcaggcctgagaagaaaacaaaaaccaaaaaaacaacatcagaggaccagagtctggggccagtgcagagcccccatgacgcgggccactccctcccagtgcaacccccagagagacaggtcttgctctcggcatctgaaaaaccactagctctcctgcccagcacccaggctgcagtatctctgggcccgtatggagcttctagaagttatgtttacctgcccacatttaacgaagagctgggtccccaacatcacctttgtctcaaaaagagcttaaaaaacaaaagcgtgggaaatccggctggacccaccttccccctgggaagttcacagatcacagattttagctcccttgctgggcaagccttcagcggctccagtccattctccactccggagagtccttgctgctgagaggctggctgggactctaggacatcagaatcgagccgcctcataactgcccctcctccactacataaccaaagcgggaagctctacctctccccagctctgcctggagacgaaggcaaattggggtattaaaagct

SEQ ID NO: 6 - protein, 348 aa, Bos taurus
MNGTEGPNFYVPFSNKTGVVRSPFEAPQYYLAEPWQFSMLAAYMFLLIMLGFPINFLTLYVTVQHKKLRTPLNYILLNLAVADLFMVFGGFTTTLYTSLHGYFVFGPTGCNLEGFFATLGGEIALWSLVVLAIERYVVVCKPMSNFRFGENHAIMGVAFTWVMALACAAPPLVGWSRYIPEGMQCSCGIDYYTPHEETNNESFVIYMFVVHFIIPLIVIFFCYGQLVFTVKEAAAQQQESATTQKAEKEVTRMVIIMVIAFLICWLPYAGVAFYIFTHQGSDFGPIFMTIPAFFAKTSAVYNPVIYIMMNKQFRNCMVTTLCCGKNPLGDDEASTTVSKTETSQVAPA